European Patent Specification EP 3 797 167 B1, published September 18, 2024. Title: A METHOD OF PRODUCING A TRIPEPTIDE GAMMA-GLU-VAL-GLY USING ENTEROBACTERIACEAE. Applicant: Ajinomoto Co., Inc. The sequence listing filed with the application follows.

SEQUENCE LISTING (64 sequences)

SEQ ID NO: 1 - DNA, 1026 bp, Escherichia coli
atgaaagcgttatccaaactgaaagcggaagagggcatctggatgaccgacgttcctgtaccggaactcgggcataacgatctgctgattaaaatccgtaaaacagccatctgcgggactgacgttcacatctataactgggatgagtggtcgcaaaaaaccatcccggtgccgatggtcgtgggccatgaatatgtcggtgaagtggtaggtattggtcaggaagtgaaaggcttcaagatcggcgatcgcgtttctggcgaaggccatatcacctgtggtcattgccgcaactgtcgtggtggtcgtacccatttgtgccgcaacacgataggcgttggtgttaatcgcccgggctgctttgccgaatatctggtgatcccggcattcaacgccttcaaaatccccgacaatatttccgatgacttagccgcaatttttgatcccttcggtaacgccgtgcataccgcgctgtcgtttgatctggtgggcgaagatgtgctggtttctggtgcaggcccgattggtattatggcagcggcggtggcgaaacacgttggtgcacgcaatgtggtgatcactgatgttaacgaataccgccttgagctggcgcgtaaaatgggtatcacccgtgcggttaacgtcgccaaagaaaatctcaatgacgtgatggcggagttaggcatgaccgaaggttttgatgtcggtctggaaatgtccggtgcgccgccagcgtttcgtaccatgcttgacaccatgaatcacggcggccgtattgcgatgctgggtattccgccgtctgatatgtctatcgactggaccaaagtgatctttaaaggcttgttcattaaaggtatttacggtcgtgagatgtttgaaacctggtacaagatggcggcgctgattcagtctggcctcgatctttcgccgatcattacccatcgtttctctatcgatgatttccagaagggctttgacgctatgcgttcgggccagtccgggaaagttattctgagctgggattaa

SEQ ID NO: 2 - protein, 341 aa, Escherichia coli
MKALSKLKAEEGIWMTDVPVPELGHNDLLIKIRKTAICGTDVHIYNWDEWSQKTIPVPMVVGHEYVGEVVGIGQEVKGFKIGDRVSGEGHITCGHCRNCRGGRTHLCRNTIGVGVNRPGCFAEYLVIPAFNAFKIPDNISDDLAAIFDPFGNAVHTALSFDLVGEDVLVSGAGPIGIMAAAVAKHVGARNVVITDVNEYRLELARKMGITRAVNVAKENLNDVMAELGMTEGFDVGLEMSGAPPAFRTMLDTMNHGGRIAMLGIPPSDMSIDWTKVIFKGLFIKGIYGREMFETWYKMAALIQSGLDLSPIITHRFSIDDFQKGFDAMRSGQSGKVILSWD

SEQ ID NO: 3 - DNA, 1197 bp, Escherichia coli
atgcgtggagaattttatcagcagttaaccaacgatctggaaaccgcacgggcggaagggttgtttaaagaagagcgcattattacgtctgcgcagcaagcagatatcactgtggctgatggaagccacgtcattaacttttgtgccaacaactatctcgggctggcgaatcatcctgatctgattgcggcggcaaaggcgggaatggattctcacggtttcggcatggcttcggtgcgttttatttgcggcactcaggacagccataaagagcttgaacaaaaactggcggccttcctggggatggaagatgcgattctctactcttcctgctttgatgctaacggtggcctgtttgaaacgcttctgggtgcggaagacgccattatctccgacgcactgaaccacgcgtctattattgatggtgtgcgtctgtgcaaagctaaacgctatcgctatgccaacaacgatatgcaggagctggaagcacgtctgaaagaagcgcgtgaagccggtgcgcgtcatgtgctgatcgccaccgatggtgtgttctcaatggacggcgtgattgccaacctgaagggcgtttgcgatctggcagataaatatgatgccctggtgatggtagacgactcccacgcggtcggttttgtcggtgaaaatggtcgtggttcccatgaatactgcgatgtgatgggccgggtcgatattatcaccggtacgcttggtaaagcgctgggcggggcttctggtggttataccgcggcgcgcaaagaagtggttgagtggctgcgccagcgttctcgtccgtacctgttctccaactcgctggcaccggccattgttgccgcgtccatcaaagtactggagatggtcgaagcgggcagcgaactgcgtgaccgtctgtgggcgaacgcgcgtcagttccgtgagcaaatgtcggcggcgggctttaccctggcgggagccgatcacgccattattccggtcatgcttggtgatgcggtagtggcgcagaaatttgcccgtgagctgcaaaaagagggcatttacgttaccggtttcttctatccggtcgttccgaaaggtcaggcgcgtattcgtacccagatgtctgcggcgcatacccctgagcaaattacgcgtgcagtagaagcatttacgcgtattggtaaacaactgggcgttatcgcctga

SEQ ID NO: 4 - protein, 398 aa, Escherichia coli
MRGEFYQQLTNDLETARAEGLFKEERIITSAQQADITVADGSHVINFCANNYLGLANHPDLIAAAKAGMDSHGFGMASVRFICGTQDSHKELEQKLAAFLGMEDAILYSSCFDANGGLFETLLGAEDAIISDALNHASIIDGVRLCKAKRYRYANNDMQELEARLKEAREAGARHVLIATDGVFSMDGVIANLKGVCDLADKYDALVMVDDSHAVGFVGENGRGSHEYCDVMGRVDIITGTLGKALGGASGGYTAARKEVVEWLRQRSRPYLFSNSLAPAIVAASIKVLEMVEAGSELRDRLWANARQFREQMSAAGFTLAGADHAIIPVMLGDAVVAQKFARELQKEGIYVTGFFYPVVPKGQARIRTQMSAAHTPEQITRAVEAFTRIGKQLGVIA

SEQ ID NO: 5 - DNA, 64 bp, Artificial Sequence
  Primer P1
aaaggatgaactacgaggaagggaacaacattcatacgctcaagttagtataaaaaagctgaac

SEQ ID NO: 6 - DNA, 70 bp, Artificial Sequence
  Primer P2
atgtaccacccactgtgcgccattcatagttagttctccttccggccaatgcttcgtttcgtatcacaca

SEQ ID NO: 7 - DNA, 1957 bp, Artificial Sequence
  DNA fragment
aaaggatgaactacgaggaagggaacaacattcatacgctcaagttagtataaaaaagctgaacgagaaacgtaaaatgatataaatatcaatatattaaattagattttgcataaaaaacagactacataatactgtaaaacacaacatatgcagtcactatgaatcaactacttagatggtattagtgacctgtaacagactgcagtggtcgaaaaaaaaagcccgcactgtcaggtgcgggcttttttctgtgttaagcttcgacgaatttctgccattcatccgcttattatcacttattcaggcgtagcaccaggcgtttaagggcaccaataactgccttaaaaaaattacgccccgccctgccactcatcgcagtactgttgtaattcattaagcattctgccgacatggaagccatcacagacggcatgatgaacctgaatcgccagcggcatcagcaccttgtcgccttgcgtataatatttgcccatggtgaaaacgggggcgaagaagttgtccatattggccacgtttaaatcaaaactggtgaaactcacccagggattggctgagacgaaaaacatattctcaataaaccctttagggaaataggccaggttttcaccgtaacacgccacatcttgcgaatatatgtgtagaaactgccggaaatcgtcgtggtattcactccagagcgatgaaaacgtttcagtttgctcatggaaaacggtgtaacaagggtgaacactatcccatatcaccagctcaccgtctttcattgccatacggaattccggatgagcattcatcaggcgggcaagaatgtgaataaaggccggataaaacttgtgcttatttttctttacggtctttaaaaaggccgtaatatccagctgaacggtctggttataggtacattgagcaactgactgaaatgcctcaaaatgttctttacgatgccattgggatatatcaacggtggtatatccagtgatttttttctccattttagcttccttagctcctgaaaatctcggatccgatatctagctagagcgcccggttgacgctgctagtgttacctagcgatttgtatcttactgcatgttacttcatgttgtcaatacctgtttttcgtgcgacttatcaggctgtctacttatccggagatccacaggacgggtgtggtcgccatgatcgcgtagtcgatagtggctccaagtagcgaagcgagcaggactgggcggcggccaaagcggtcggacagtgctccgagaacgggtgcgcatagaaattgcatcaacgcatatagcgctagcagcacgccatagtgactggcgatgctgtcggaatggacgatatcccgcaagaggcccggcagtaccggcataaccaagcctatgcctacagcatccagggtgacggtgccgaggatgacgatgagcgcattgttagatttcatacacggtgcctgactgcgttagcaatttaactgtgataaactaccgcattaaagcttatcgatgataagctgtcaaacatgagaattcgaaatcaaataatgattttattttgactgatagtgacctgttcgttgcaacaaattgataagcaatgcttttttataatgccaacttagtataaaaaagcaggcttcaagatcttcacctaccaaacaatgcccccctgcaaaaaataaattcatataaaaaacatacagataaccatctgcggtgataaattatctctggcggtgttgacataaataccactggcggtgatactgagcacatcagcaggacgcactgaccaccatgaaggtgacgctcttaaaaattaagccctgaagaagggcagcattcaaagcagaaggctttggggtgtgtgatacgaaacgaagcattggccggaaggagaactaactatgaatggcgcacagtgggtggtacat

SEQ ID NO: 8 - DNA, 22 bp, Artificial Sequence
  Primer P3
tgcaagtgaagttgagttgttc

SEQ ID NO: 9 - DNA, 21 bp, Artificial Sequence
  Primer P4
gataaccgaaaacggtgttca

SEQ ID NO: 10 - DNA, 566 bp, Artificial Sequence
  DNA fragment
tgcaagtgaagttgagttgttctggcggtggaatgatgctcgcaaaaatgcagcggacaaaggatgaactacgaggaagggaacaacattcatactgaaattgaatttttttcactcactattttatttttaaaaaacaacaatttatattgaaattattaaacgcatcataaaaatcggccaaaaaatatcttgtactatttacaaaacctatggtaactctttaggcattccttcgaacaagatgcaagaaaagacaaaatgacagcccttctacgagtgattagcctggtcgtgattagcgtggtggtgattattatcccaccgtgcggggctgcacttggacgaggaaaggcttagagatcaagccttaacgaactaagacccccgcaccgaaaggtccgggggttttttttgaccttaaaaacataaccgaggagcagacaatgaataacagcacaaaattctgtttctcaagattcaggacggggaactaactatgaatggcgcacagtgggtggtacatgcgttgcgggcacagggtgtgaacaccgttttcggttatc

SEQ ID NO: 11 - DNA, 2055 bp, Artificial Sequence
  DNA fragment
tgcaagtgaagttgagttgttctggcggtggaatgatgctcgcaaaaatgcagcggacaaaggatgaactacgaggaagggaacaacattcatacgctcaagttagtataaaaaagctgaacgagaaacgtaaaatgatataaatatcaatatattaaattagattttgcataaaaaacagactacataatactgtaaaacacaacatatgcagtcactatgaatcaactacttagatggtattagtgacctgtaacagactgcagtggtcgaaaaaaaaagcccgcactgtcaggtgcgggcttttttctgtgttaagcttcgacgaatttctgccattcatccgcttattatcacttattcaggcgtagcaccaggcgtttaagggcaccaataactgccttaaaaaaattacgccccgccctgccactcatcgcagtactgttgtaattcattaagcattctgccgacatggaagccatcacagacggcatgatgaacctgaatcgccagcggcatcagcaccttgtcgccttgcgtataatatttgcccatggtgaaaacgggggcgaagaagttgtccatattggccacgtttaaatcaaaactggtgaaactcacccagggattggctgagacgaaaaacatattctcaataaaccctttagggaaataggccaggttttcaccgtaacacgccacatcttgcgaatatatgtgtagaaactgccggaaatcgtcgtggtattcactccagagcgatgaaaacgtttcagtttgctcatggaaaacggtgtaacaagggtgaacactatcccatatcaccagctcaccgtctttcattgccatacggaattccggatgagcattcatcaggcgggcaagaatgtgaataaaggccggataaaacttgtgcttatttttctttacggtctttaaaaaggccgtaatatccagctgaacggtctggttataggtacattgagcaactgactgaaatgcctcaaaatgttctttacgatgccattgggatatatcaacggtggtatatccagtgatttttttctccattttagcttccttagctcctgaaaatctcggatccgatatctagctagagcgcccggttgacgctgctagtgttacctagcgatttgtatcttactgcatgttacttcatgttgtcaatacctgtttttcgtgcgacttatcaggctgtctacttatccggagatccacaggacgggtgtggtcgccatgatcgcgtagtcgatagtggctccaagtagcgaagcgagcaggactgggcggcggccaaagcggtcggacagtgctccgagaacgggtgcgcatagaaattgcatcaacgcatatagcgctagcagcacgccatagtgactggcgatgctgtcggaatggacgatatcccgcaagaggcccggcagtaccggcataaccaagcctatgcctacagcatccagggtgacggtgccgaggatgacgatgagcgcattgttagatttcatacacggtgcctgactgcgttagcaatttaactgtgataaactaccgcattaaagcttatcgatgataagctgtcaaacatgagaattcgaaatcaaataatgattttattttgactgatagtgacctgttcgttgcaacaaattgataagcaatgcttttttataatgccaacttagtataaaaaagcaggcttcaagatcttcacctaccaaacaatgcccccctgcaaaaaataaattcatataaaaaacatacagataaccatctgcggtgataaattatctctggcggtgttgacataaataccactggcggtgatactgagcacatcagcaggacgcactgaccaccatgaaggtgacgctcttaaaaattaagccctgaagaagggcagcattcaaagcagaaggctttggggtgtgtgatacgaaacgaagcattggccggaaggagaactaactatgaatggcgcacagtgggtggtacatgcgttgcgggcacagggtgtgaacaccgttttcggttatc

SEQ ID NO: 12 - DNA, 20 bp, Artificial Sequence
  Primer P5
gctaagggctaatgagttat

SEQ ID NO: 13 - DNA, 20 bp, Artificial Sequence
  Primer P6
ctcaaaagcagtcaagagtg

SEQ ID NO: 14 - DNA, 1850 bp, Artificial Sequence
  PCR product
gctaagggctaatgagttatatgcaaattagtaaaattatgttgctatgtcagatagttacgatttagtcatctaactatgaagcctgcttttttatactaagttggcattataaaaaagcattgcttatcaatttgttgcaacgaacaggtcactatcagtcaaaataaaatcattatttgatttcgaattccccggatccgtcgacctgcaggggggggggggcgctgaggtctgcctcgtgaagaaggtgttgctgactcataccaggcctgaatcgccccatcatccagccagaaagtgagggagccacggttgatgagagctttgttgtaggtggaccagttggtgattttgaacttttgctttgccacggaacggtctgcgttgtcgggaagatgcgtgatctgatccttcaactcagcaaaagttcgatttattcaacaaagccgccgtcccgtcaagtcagcgtaatgctctgccagtgttacaaccaattaaccaattctgattagaaaaactcatcgagcatcaaatgaaactgcaatttattcatatcaggattatcaataccatatttttgaaaaagccgtttctgtaatgaaggagaaaactcaccgaggcagttccataggatggcaagatcctggtatcggtctgcgattccgactcgtccaacatcaatacaacctattaatttcccctcgtcaaaaataaggttatcaagtgagaaatcaccatgagtgacgactgaatccggtgagaatggcaaaagcttatgcatttctttccagacttgttcaacaggccagccattacgctcgtcatcaaaatcactcgcatcaaccaaaccgttattcattcgtgattgcgcctgagcgagacgaaatacgcgatcgctgttaaaaggacaattacaaacaggaatcgaatgcaaccggcgcaggaacactgccagcgcatcaacaatattttcacctgaatcaggatattcttctaatacctggaatgctgttttcccggggatcgcagtggtgagtaaccatgcatcatcaggagtacggataaaatgcttgatggtcggaagaggcataaattccgtcagccagtttagtctgaccatctcatctgtaacatcattggcaacgctacctttgccatgtttcagaaacaactctggcgcatcgggcttcccatacaatcgatagattgtcgcacctgattgcccgacattatcgcgagcccatttatacccatataaatcagcatccatgttggaatttaatcgcggcctcgagcaagacgtttcccgttgaatatggctcataacaccccttgtattactgtttatgtaagcagacagttttattgttcatgatgatatatttttatcttgtgcaatgtaacatcagagattttgagacacaacgtggctttcccccccccccctgcagtctgttacaggtcactaataccatctaagtagttgattcatagtgactgcatatgttgtgttttacagtattatgtagtctgttttttatgcaaaatctaatttaatatattgatatttatatcattttacgtttctcgttcagcttttttatactaacttgagcgtctagccctgttgacaattaatcatcggctcgtataatgtgtggaatcgtgagcggataacaatttcacacaaataattttgtttaactttaagaaggagatataatgatcccggacgtatcacaggcgctggcctggctggaaaaacatcctcaggcgttaaaggggatacagcgtgggctggagcgcgaaactttgcgtgttaatgctgatggcacactggcaacaac

SEQ ID NO: 15 - DNA, 64 bp, Artificial Sequence
  Primer P9
ctactatctgtaggtgttgagagacatcaagttacacgctcaagttagtataaaaaagctgaac

SEQ ID NO: 16 - DNA, 64 bp, Artificial Sequence
  Primer P10
cagatcgttggttaactgctgataaaattctccacgcatagttagttctccttccggccaatgc

SEQ ID NO: 17 - DNA, 1969 bp, Artificial Sequence
  PCR product
ctactatctgtaggtgttgagagacatcaagttacacgctcaagttagtataaaaaagctgaacgagaaacgtaaaatgatataaatatcaatatattaaattagattttgcataaaaaacagactacataatactgtaaaacacaacatatgcagtcactatgaatcaactacttagatggtattagtgacctgtaacagactgcagtggtcgaaaaaaaaagcccgcactgtcaggtgcgggcttttttctgtgttaagcttcgacgaatttctgccattcatccgcttattatcacttattcaggcgtagcaccaggcgtttaagggcaccaataactgccttaaaaaaattacgccccgccctgccactcatcgcagtactgttgtaattcattaagcattctgccgacatggaagccatcacagacggcatgatgaacctgaatcgccagcggcatcagcaccttgtcgccttgcgtataatatttgcccatggtgaaaacgggggcgaagaagttgtccatattggccacgtttaaatcaaaactggtgaaactcacccagggattggctgagacgaaaaacatattctcaataaaccctttagggaaataggccaggttttcaccgtaacacgccacatcttgcgaatatatgtgtagaaactgccggaaatcgtcgtggtattcactccagagcgatgaaaacgtttcagtttgctcatggaaaacggtgtaacaagggtgaacactatcccatatcaccagctcaccgtctttcattgccatacggaattccggatgagcattcatcaggcgggcaagaatgtgaataaaggccggataaaacttgtgcttatttttctttacggtctttaaaaaggccgtaatatccagctgaacggtctggttataggtacattgagcaactgactgaaatgcctcaaaatgttctttacgatgccattgggatatatcaacggtggtatatccagtgatttttttctccattttagcttccttagctcctgaaaatctcggatccgatatctagctagagcgcccggttgacgctgctagtgttacctagcgatttgtatcttactgcatgttacttcatgttgtcaatacctgtttttcgtgcgacttatcaggctgtctacttatccggagatccacaggacgggtgtggtcgccatgatcgcgtagtcgatagtggctccaagtagcgaagcgagcaggactgggcggcggccaaagcggtcggacagtgctccgagaacgggtgcgcatagaaattgcatcaacgcatatagcgctagcagcacgccatagtgactggcgatgctgtcggaatggacgatatcccgcaagaggcccggcagtaccggcataaccaagcctatgcctacagcatccagggtgacggtgccgaggatgacgatgagcgcattgttagatttcatacacggtgcctgactgcgttagcaatttaactgtgataaactaccgcattaaagcttatcgatgataagctgtcaaacatgagaattcgaaatcaaataatgattttattttgactgatagtgacctgttcgttgcaacaaattgataagcaatgcttttttataatgccaacttagtataaaaaagcaggcttcaagatcttcacctaccaaacaatgcccccctgcaaaaaataaattcatataaaaaacatacagataaccatctgcggtgataaattatctctggcggtgttgacataaataccactggcggtgatactgagcacatcagcaggacgcactgaccaccatgaaggtgacgctcttaaaaattaagccctgaagaagggcagcattcaaagcagaaggctttggggtgtgtgatacgaaacgaagcattggccggaaggagaactaactatgcgtggagaattttatcagcagttaaccaacgatctg

SEQ ID NO: 18 - DNA, 20 bp, Artificial Sequence
  Primer P11
cctccattagtgggtagcgt

SEQ ID NO: 19 - DNA, 20 bp, Artificial Sequence
  Primer P12
agaatccattcccgcctttg

SEQ ID NO: 20 - DNA, 482 bp, Artificial Sequence
  PCR product
cctccattagtgggtagcgttttgataccaactgagataggaaaaatgatgctttggcatcattttttctttttatatcaatgcagtaaaatcaatcatcattatgcccagccaaaactgtacagtttttctactatctgtaggtgttgagagacatcaagttacacgttatttatcctgaattttgcagaagtgttaacgcgttatctcgtcgcgacctataagtttgggtaatatgtgctggaatttgccctgtctggagaatcgcaatgcgtggagaattttatcagcagttaaccaacgatctggaaaccgcacgggcggaagggttgtttaaagaagagcgcattattacgtctgcgcagcaagcagatatcactgtggctgatggaagccacgtcattaacttttgtgccaacaactatctcgggctggcgaatcatcctgatctgattgcggcggcaaaggcgggaatggattct

SEQ ID NO: 21 - DNA, 2273 bp, Artificial Sequence
  PCR product
cctccattagtgggtagcgttttgataccaactgagataggaaaaatgatgctttggcatcattttttctttttatatcaatgcagtaaaatcaatcatcattatgcccagccaaaactgtacagtttttctactatctgtaggtgttgagagacatcaagttacacgctcaagttagtataaaaaagctgaacgagaaacgtaaaatgatataaatatcaatatattaaattagattttgcataaaaaacagactacataatactgtaaaacacaacatatgcagtcactatgaatcaactacttagatggtattagtgacctgtaacagactgcagtggtcgaaaaaaaaagcccgcactgtcaggtgcgggcttttttctgtgttaagcttcgacgaatttctgccattcatccgcttattatcacttattcaggcgtagcaccaggcgtttaagggcaccaataactgccttaaaaaaattacgccccgccctgccactcatcgcagtactgttgtaattcattaagcattctgccgacatggaagccatcacagacggcatgatgaacctgaatcgccagcggcatcagcaccttgtcgccttgcgtataatatttgcccatggtgaaaacgggggcgaagaagttgtccatattggccacgtttaaatcaaaactggtgaaactcacccagggattggctgagacgaaaaacatattctcaataaaccctttagggaaataggccaggttttcaccgtaacacgccacatcttgcgaatatatgtgtagaaactgccggaaatcgtcgtggtattcactccagagcgatgaaaacgtttcagtttgctcatggaaaacggtgtaacaagggtgaacactatcccatatcaccagctcaccgtctttcattgccatacggaattccggatgagcattcatcaggcgggcaagaatgtgaataaaggccggataaaacttgtgcttatttttctttacggtctttaaaaaggccgtaatatccagctgaacggtctggttataggtacattgagcaactgactgaaatgcctcaaaatgttctttacgatgccattgggatatatcaacggtggtatatccagtgatttttttctccattttagcttccttagctcctgaaaatctcggatccgatatctagctagagcgcccggttgacgctgctagtgttacctagcgatttgtatcttactgcatgttacttcatgttgtcaatacctgtttttcgtgcgacttatcaggctgtctacttatccggagatccacaggacgggtgtggtcgccatgatcgcgtagtcgatagtggctccaagtagcgaagcgagcaggactgggcggcggccaaagcggtcggacagtgctccgagaacgggtgcgcatagaaattgcatcaacgcatatagcgctagcagcacgccatagtgactggcgatgctgtcggaatggacgatatcccgcaagaggcccggcagtaccggcataaccaagcctatgcctacagcatccagggtgacggtgccgaggatgacgatgagcgcattgttagatttcatacacggtgcctgactgcgttagcaatttaactgtgataaactaccgcattaaagcttatcgatgataagctgtcaaacatgagaattcgaaatcaaataatgattttattttgactgatagtgacctgttcgttgcaacaaattgataagcaatgcttttttataatgccaacttagtataaaaaagcaggcttcaagatcttcacctaccaaacaatgcccccctgcaaaaaataaattcatataaaaaacatacagataaccatctgcggtgataaattatctctggcggtgttgacataaataccactggcggtgatactgagcacatcagcaggacgcactgaccaccatgaaggtgacgctcttaaaaattaagccctgaagaagggcagcattcaaagcagaaggctttggggtgtgtgatacgaaacgaagcattggccggaaggagaactaactatgcgtggagaattttatcagcagttaaccaacgatctggaaaccgcacgggcggaagggttgtttaaagaagagcgcattattacgtctgcgcagcaagcagatatcactgtggctgatggaagccacgtcattaacttttgtgccaacaactatctcgggctggcgaatcatcctgatctgattgcggcggcaaaggcgggaatggattct

SEQ ID NO: 22 - DNA, 65 bp, Artificial Sequence
  Primer P13
gttcacaattcactgcacgtttcaggaaccatcgctccgctcaagttagtataaaaaagctgaac

SEQ ID NO: 23 - DNA, 64 bp, Artificial Sequence
  Primer P14
gccgaagcgcctttagaaaatagtcgaatcagtgaatgaagcctgcttttttatactaagttgg

SEQ ID NO: 24 - DNA, 1614 bp, Artificial Sequence
  PCR product
gttcacaattcactgcacgtttcaggaaccatcgctccgctcaagttagtataaaaaagctgaacgagaaacgtaaaatgatataaatatcaatatattaaattagattttgcataaaaaacagactacataatactgtaaaacacaacatatgcagtcactatgaatcaactacttagatggtattagtgacctgtaacagactgcaggggggggggggaaagccacgttgtgtctcaaaatctctgatgttacattgcacaagataaaaatatatcatcatgaacaataaaactgtctgcttacataaacagtaatacaaggggtgttatgagccatattcaacgggaaacgtcttgctcgaggccgcgattaaattccaacatggatgctgatttatatgggtataaatgggctcgcgataatgtcgggcaatcaggtgcgacaatctatcgattgtatgggaagcccgatgcgccagagttgtttctgaaacatggcaaaggtagcgttgccaatgatgttacagatgagatggtcagactaaactggctgacggaatttatgcctcttccgaccatcaagcattttatccgtactcctgatgatgcatggttactcaccactgcgatccccgggaaaacagcattccaggtattagaagaatatcctgattcaggtgaaaatattgttgatgcgctggcagtgttcctgcgccggttgcattcgattcctgtttgtaattgtccttttaacagcgatcgcgtatttcgtctcgctcaggcgcaatcacgaatgaataacggtttggttgatgcgagtgattttgatgacgagcgtaatggctggcctgttgaacaagtctggaaagaaatgcataagcttttgccattctcaccggattcagtcgtcactcatggtgatttctcacttgataaccttatttttgacgaggggaaattaataggttgtattgatgttggacgagtcggaatcgcagaccgataccaggatcttgccatcctatggaactgcctcggtgagttttctccttcattacagaaacggctttttcaaaaatatggtattgataatcctgatatgaataaattgcagtttcatttgatgctcgatgagtttttctaatcagaattggttaattggttgtaacactggcagagcattacgctgacttgacgggacggcggctttgttgaataaatcgaacttttgctgagttgaaggatcagatcacgcatcttcccgacaacgcagaccgttccgtggcaaagcaaaagttcaaaatcaccaactggtccacctacaacaaagctctcatcaaccgtggctccctcactttctggctggatgatggggcgattcaggcctggtatgagtcagcaacaccttcttcacgaggcagacctcagcgcccccccccccctgcaggtcgacggatccggggaattcgaaatcaaataatgattttattttgactgatagtgacctgttcgttgcaacaaattgataagcaatgcttttttataatgccaacttagtataaaaaagcaggcttcattcactgattcgactattttctaaaggcgcttcggc

SEQ ID NO: 25 - DNA, 20 bp, Artificial Sequence
  Primer P15
cggctttattcctcttctgc

SEQ ID NO: 26 - DNA, 20 bp, Artificial Sequence
  Primer P16
taaatattcgcgccagtgcc

SEQ ID NO: 27 - DNA, 3136 bp, Artificial Sequence
  PCR product
cggctttattcctcttctgcgggagaggatcagggtgaggaaaatttatgcctcaccctcactctcttcgtaaggagagaggttcacaattcactgcacgtttcaggaaccatcgctcatgacacagacgttaagccagcttgaaaacagcggcgcttttattgaacgccatatcggaccggacgccgcgcaacagcaagaaatgctgaatgccgttggtgcacaatcgttaaacgcgctgaccggccagattgtgccgaaagatattcaacttgcgacaccaccgcaggttggcgcaccggcgaccgaatacgccgcactggcagaactcaaggctattgccagtcgcaataaacgcttcacgtcttacatcggcatgggttacaccgccgtgcagctaccgccggttatcctgcgtaacatgctggaaaatccgggctggtataccgcgtacactccgtatcaacctgaagtctcccagggccgccttgaagcactgctcaacttccagcaggtaacgctggatttgactggactggatatggcctctgcttctcttctggacgaggccaccgctgccgccgaagcaatggcgatggcgaaacgcgtcagcaaactgaaaaatgccaaccgcttcttcgtggcttccgatgtgcatccgcaaacgctggatgtggtccgtactcgtgccgaaacctttggttttgaagtgattgtcgatgacgcgcaaaaagtgctcgaccatcaggacgtcttcggcgtgctgttacagcaggtaggcactaccggtgaaattcacgactacactgcgcttattagcgaactgaaatcacgcaaaattgtggtcagcgttgccgccgatattatggcgctggtgctgttaactgcgccgggtaaacagggcgcggatattgtttttggttcggcgcaacgcttcggcgtgccgatgggctacggtggcccacacgcggcattctttgcggcgaaagatgaatacaaacgctcaatgccgggccgtattatcggtgtatcgaaagatgcagctggcaataccgcgctgcgcatggcgatgcagactcgcgagcaacatatccgccgtgagaaagcgaactccaacatttgtacttcccaggtactgctggcaaacatcgccagcctgtatgccgtttatcacggcccggttggcctgaaacgtatcgctaaccgcattcaccgtctgaccgatatcctggcggcgggcctgcaacaaaaaggtctgaaactgcgccatgcgcactatttcgacaccttgtgtgtggaagtggccgacaaagcgggcgtactgacgcgtgccgaagcggctgaaatcaacctgcgtagcgatattctgaacgcggttgggatcacccttgatgaaacaaccacgcgtgaaaacgtaatgcagcttttcaacgtgctgctgggcgataaccacggcctggacatcgacacgctggacaaagacgtggctcacgacagccgctctatccagcctgcgatgctgcgcgacgacgaaatcctcacccatccggtgtttaatcgctaccacagcgaaaccgaaatgatgcgctatatgcactcgctggagcgtaaagatctggcgctgaatcaggcgatgatcccgctgggttcctgcaccatgaaactgaacgccgccgccgagatgatcccaatcacctggccggaatttgccgaactgcacccgttctgcccgccggagcaggccgaaggttatcagcagatgattgcgcagctggctgactggctggtgaaactgaccggttacgacgccgtttgtatgcagccgaactctggcgcacagggcgaatacgcgggcctgctggcgattcgtcattatcatgaaagccgcaacgaagggcatcgcgatatctgcctgatcccggcttctgcgcacggaactaaccccgcttctgcacatatggcaggaatgcaggtggtggttgtggcgtgtgataaaaacggcaacatcgatctgactgatctgcgcgcgaaagcggaacaggcgggcgataacctctcctgtatcatggtgacttatccttctacccacggcgtgtatgaagaaacgatccgtgaagtgtgtgaagtcgtgcatcagttcggcggtcaggtttaccttgatggcgcgaacatgaacgcccaggttggcatcacctcgccgggctttattggtgcggacgtttcacaccttaacctacataaaactttctgcattccgcacggcggtggtggtccgggtatgggaccgatcggcgtgaaagcgcatttggcaccgtttgtaccgggtcatagcgtggtgcaaatcgaaggcatgttaacccgtcagggcgcggtttctgcggcaccgttcggtagcgcctctatcctgccaatcagctggatgtacatccgcatgatgggcgcagaagggctgaaaaaagcaagccaggtggcaatcctcaacgccaactatattgccagccgcctgcaggatgccttcccggtgctgtataccggtcgcgacggtcgcgtggcgcacgaatgtattctcgatattcgcccgctgaaagaagaaaccggcatcagcgagctggatattgccaagcgcctgatcgactacggtttccacgcgccgacgatgtcgttcccggtggcgggtacgctgatggttgaaccgactgaatctgaaagcaaagtggaactggatcgctttatcgacgcgatgctggctatccgcgcagaaattgaccaggtgaaagccggtgtctggccgctggaagataacccgctggtgaacgcgccgcacattcagagcgaactggtcgccgagtgggcgcatccgtacagccgtgaagttgcggtattcccggcaggtgtggcagacaaatactggccgacagtgaaacgtctggatgatgtttacggcgaccgtaacctgttctgctcctgcgtaccgattagcgaataccagtaattcactgattcgactattttctaaaggcgcttcggcgcctttttagtcagatgacaaagtacaaaagtgctcagacagtcccctcgcccctttggggagagggttagggtgaggggaacaggccggcactggcgcgaatattta

SEQ ID NO: 28 - DNA, 1803 bp, Artificial Sequence
  PCR product
cggctttattcctcttctgcgggagaggatcagggtgaggaaaatttatgcctcaccctcactctcttcgtaaggagagaggttcacaattcactgcacgtttcaggaaccatcgctccgctcaagttagtataaaaaagctgaacgagaaacgtaaaatgatataaatatcaatatattaaattagattttgcataaaaaacagactacataatactgtaaaacacaacatatgcagtcactatgaatcaactacttagatggtattagtgacctgtaacagactgcaggggggggggggaaagccacgttgtgtctcaaaatctctgatgttacattgcacaagataaaaatatatcatcatgaacaataaaactgtctgcttacataaacagtaatacaaggggtgttatgagccatattcaacgggaaacgtcttgctcgaggccgcgattaaattccaacatggatgctgatttatatgggtataaatgggctcgcgataatgtcgggcaatcaggtgcgacaatctatcgattgtatgggaagcccgatgcgccagagttgtttctgaaacatggcaaaggtagcgttgccaatgatgttacagatgagatggtcagactaaactggctgacggaatttatgcctcttccgaccatcaagcattttatccgtactcctgatgatgcatggttactcaccactgcgatccccgggaaaacagcattccaggtattagaagaatatcctgattcaggtgaaaatattgttgatgcgctggcagtgttcctgcgccggttgcattcgattcctgtttgtaattgtccttttaacagcgatcgcgtatttcgtctcgctcaggcgcaatcacgaatgaataacggtttggttgatgcgagtgattttgatgacgagcgtaatggctggcctgttgaacaagtctggaaagaaatgcataagcttttgccattctcaccggattcagtcgtcactcatggtgatttctcacttgataaccttatttttgacgaggggaaattaataggttgtattgatgttggacgagtcggaatcgcagaccgataccaggatcttgccatcctatggaactgcctcggtgagttttctccttcattacagaaacggctttttcaaaaatatggtattgataatcctgatatgaataaattgcagtttcatttgatgctcgatgagtttttctaatcagaattggttaattggttgtaacactggcagagcattacgctgacttgacgggacggcggctttgttgaataaatcgaacttttgctgagttgaaggatcagatcacgcatcttcccgacaacgcagaccgttccgtggcaaagcaaaagttcaaaatcaccaactggtccacctacaacaaagctctcatcaaccgtggctccctcactttctggctggatgatggggcgattcaggcctggtatgagtcagcaacaccttcttcacgaggcagacctcagcgcccccccccccctgcaggtcgacggatccggggaattcgaaatcaaataatgattttattttgactgatagtgacctgttcgttgcaacaaattgataagcaatgcttttttataatgccaacttagtataaaaaagcaggcttcattcactgattcgactattttctaaaggcgcttcggcgcctttttagtcagatgacaaagtacaaaagtgctcagacagtcccctcgcccctttggggagagggttagggtgaggggaacaggccggcactggcgcgaatattta

SEQ ID NO: 29 - DNA, 458 bp, Artificial Sequence
  PCR product
tgcaagtgaagttgagttgttctggcggtggaatgatgctcgcaaaaatgcagcggacaaaggatgaactacgaggaagggaacaacattcatacgctcaagttagtataaaaaagcaggcttcaagatcttcacctaccaaacaatgcccccctgcaaaaaataaattcatataaaaaacatacagataaccatctgcggtgataaattatctctggcggtgttgacataaataccactggcggtgatactgagcacatcagcaggacgcactgaccaccatgaaggtgacgctcttaaaaattaagccctgaagaagggcagcattcaaagcagaaggctttggggtgtgtgatacgaaacgaagcattggccggaaggagaactaactatgaatggcgcacagtgggtggtacatgcgttgcgggcacagggtgtgaacaccgttttcggttatc

SEQ ID NO: 30 - DNA, 64 bp, Artificial Sequence
  Primer P17
ggccagtgccaagcttgcatgcctgcaggtcgactctgaagcctgcttttttatactaagttgg

SEQ ID NO: 31 - DNA, 64 bp, Artificial Sequence
  Primer P18
gtttgcgatggggtccatcacgatgccgagcttgatcattatatctccttcttaaagttaaaca

SEQ ID NO: 32 - DNA, 1721 bp, Artificial Sequence
  PCR product
ggccagtgccaagcttgcatgcctgcaggtcgactctgaagcctgcttttttatactaagttggcattataaaaaagcattgcttatcaatttgttgcaacgaacaggtcactatcagtcaaaataaaatcattatttgatttcgaattccccggatccgtcgacctgcaggggggggggggcgctgaggtctgcctcgtgaagaaggtgttgctgactcataccaggcctgaatcgccccatcatccagccagaaagtgagggagccacggttgatgagagctttgttgtaggtggaccagttggtgattttgaacttttgctttgccacggaacggtctgcgttgtcgggaagatgcgtgatctgatccttcaactcagcaaaagttcgatttattcaacaaagccgccgtcccgtcaagtcagcgtaatgctctgccagtgttacaaccaattaaccaattctgattagaaaaactcatcgagcatcaaatgaaactgcaatttattcatatcaggattatcaataccatatttttgaaaaagccgtttctgtaatgaaggagaaaactcaccgaggcagttccataggatggcaagatcctggtatcggtctgcgattccgactcgtccaacatcaatacaacctattaatttcccctcgtcaaaaataaggttatcaagtgagaaatcaccatgagtgacgactgaatccggtgagaatggcaaaagcttatgcatttctttccagacttgttcaacaggccagccattacgctcgtcatcaaaatcactcgcatcaaccaaaccgttattcattcgtgattgcgcctgagcgagacgaaatacgcgatcgctgttaaaaggacaattacaaacaggaatcgaatgcaaccggcgcaggaacactgccagcgcatcaacaatattttcacctgaatcaggatattcttctaatacctggaatgctgttttcccggggatcgcagtggtgagtaaccatgcatcatcaggagtacggataaaatgcttgatggtcggaagaggcataaattccgtcagccagtttagtctgaccatctcatctgtaacatcattggcaacgctacctttgccatgtttcagaaacaactctggcgcatcgggcttcccatacaatcgatagattgtcgcacctgattgcccgacattatcgcgagcccatttatacccatataaatcagcatccatgttggaatttaatcgcggcctcgagcaagacgtttcccgttgaatatggctcataacaccccttgtattactgtttatgtaagcagacagttttattgttcatgatgatatatttttatcttgtgcaatgtaacatcagagattttgagacacaacgtggctttcccccccccccctgcagtctgttacaggtcactaataccatctaagtagttgattcatagtgactgcatatgttgtgttttacagtattatgtagtctgttttttatgcaaaatctaatttaatatattgatatttatatcattttacgtttctcgttcagcttttttatactaacttgagcgtctagccctgttgacaattaatcatcggctcgtataatgtgtggaatcgtgagcggataacaatttcacacaaataattttgtttaactttaagaaggagatataatgatcaagctcggcatcgtgatggaccccatcgcaaac

SEQ ID NO: 33 - DNA, 20 bp, Artificial Sequence
  Primer P7
ctgagtaggacaaatccgcc

SEQ ID NO: 34 - DNA, 20 bp, Artificial Sequence
  Primer P8
accacgacgctgtgcttcca

SEQ ID NO: 35 - DNA, 274 bp, Artificial Sequence
  PCR product
ctgagtaggacaaatccgccgggagcggatttgaacgttgcgaagcaacggcccggagggtggcgggcaggacgcccgccataaactgccaggcatcaaattaagcagaaggccatcctgacggatggcctttttgcgtggccagtgccaagcttgcatgcctgcaggtcgactctagatgatcaagctcggcatcgtgatggaccccatcgcaaacatcaacatcaagaaagattccagttttgctatgttgctggaagcacagcgtcgtggt

SEQ ID NO: 36 - DNA, 1917 bp, Artificial Sequence
  PCR product
ctgagtaggacaaatccgccgggagcggatttgaacgttgcgaagcaacggcccggagggtggcgggcaggacgcccgccataaactgccaggcatcaaattaagcagaaggccatcctgacggatggcctttttgcgtggccagtgccaagcttgcatgcctgcaggtcgactctgaagcctgcttttttatactaagttggcattataaaaaagcattgcttatcaatttgttgcaacgaacaggtcactatcagtcaaaataaaatcattatttgatttcgaattccccggatccgtcgacctgcaggggggggggggcgctgaggtctgcctcgtgaagaaggtgttgctgactcataccaggcctgaatcgccccatcatccagccagaaagtgagggagccacggttgatgagagctttgttgtaggtggaccagttggtgattttgaacttttgctttgccacggaacggtctgcgttgtcgggaagatgcgtgatctgatccttcaactcagcaaaagttcgatttattcaacaaagccgccgtcccgtcaagtcagcgtaatgctctgccagtgttacaaccaattaaccaattctgattagaaaaactcatcgagcatcaaatgaaactgcaatttattcatatcaggattatcaataccatatttttgaaaaagccgtttctgtaatgaaggagaaaactcaccgaggcagttccataggatggcaagatcctggtatcggtctgcgattccgactcgtccaacatcaatacaacctattaatttcccctcgtcaaaaataaggttatcaagtgagaaatcaccatgagtgacgactgaatccggtgagaatggcaaaagcttatgcatttctttccagacttgttcaacaggccagccattacgctcgtcatcaaaatcactcgcatcaaccaaaccgttattcattcgtgattgcgcctgagcgagacgaaatacgcgatcgctgttaaaaggacaattacaaacaggaatcgaatgcaaccggcgcaggaacactgccagcgcatcaacaatattttcacctgaatcaggatattcttctaatacctggaatgctgttttcccggggatcgcagtggtgagtaaccatgcatcatcaggagtacggataaaatgcttgatggtcggaagaggcataaattccgtcagccagtttagtctgaccatctcatctgtaacatcattggcaacgctacctttgccatgtttcagaaacaactctggcgcatcgggcttcccatacaatcgatagattgtcgcacctgattgcccgacattatcgcgagcccatttatacccatataaatcagcatccatgttggaatttaatcgcggcctcgagcaagacgtttcccgttgaatatggctcataacaccccttgtattactgtttatgtaagcagacagttttattgttcatgatgatatatttttatcttgtgcaatgtaacatcagagattttgagacacaacgtggctttcccccccccccctgcagtctgttacaggtcactaataccatctaagtagttgattcatagtgactgcatatgttgtgttttacagtattatgtagtctgttttttatgcaaaatctaatttaatatattgatatttatatcattttacgtttctcgttcagcttttttatactaacttgagcgtctagccctgttgacaattaatcatcggctcgtataatgtgtggaatcgtgagcggataacaatttcacacaaataattttgtttaactttaagaaggagatataatgatcaagctcggcatcgtgatggaccccatcgcaaacatcaacatcaagaaagattccagttttgctatgttgctggaagcacagcgtcgtggt

SEQ ID NO: 37 - DNA, 64 bp, Artificial Sequence
  Primer P19
cagagcacaaccacatcacaacaaatccgcgcctgatgaagcctgcttttttatactaagttgg

SEQ ID NO: 38 - DNA, 64 bp, Artificial Sequence
  Primer P20
catactttatttactcccagtgtctgtctcgtaaatcgctcaagttagtataaaaaagctgaac

SEQ ID NO: 39 - DNA, 1713 bp, Artificial Sequence
  PCR product
cagagcacaaccacatcacaacaaatccgcgcctgatgaagcctgcttttttatactaagttggcattataaaaaagcattgcttatcaatttgttgcaacgaacaggtcactatcagtcaaaataaaatcattatttgatttcgaattctcatgtttgacagcttatcatcgataagctttaatgcggtagtttatcacagttaaattgctaacgcagtcaggcaccgtgtatgaaatctaacaatgcgctcatcgtcatcctcggcaccgtcaccctggatgctgtaggcataggcttggttatgccggtactgccgggcctcttgcgggatatcgtccattccgacagcatcgccagtcactatggcgtgctgctagcgctatatgcgttgatgcaatttctatgcgcacccgttctcggagcactgtccgaccgctttggccgccgcccagtcctgctcgcttcgctacttggagccactatcgactacgcgatcatggcgaccacacccgtcctgtggatctccggataagtagacagcctgataagtcgcacgaaaaacaggtattgacaacatgaagtaacatgcagtaagatacaaatcgctaggtaacactagcagcgtcaaccgggcgctctagctagagccaagctagcttggccggatccgagattttcaggagctaaggaagctaaaatggagaaaaaaatcactggatataccaccgttgatatatcccaatggcatcgtaaagaacattttgaggcatttcagtcagttgctcaatgtacctataaccagaccgttcagctggatattacggcctttttaaagaccgtaaagaaaaataagcacaagttttatccggcctttattcacattcttgcccgcctgatgaatgctcatccggaattccgtatggcaatgaaagacggtgagctggtgatatgggatagtgttcacccttgttacaccgttttccatgagcaaactgaaacgttttcatcgctctggagtgaataccacgacgatttccggcagtttctacacatatattcgcaagatgtggcgtgttacggtgaaaacctggcctatttccctaaagggtttattgagaatatgtttttcgtctcagccaatccctgggtgagtttcaccagttttgatttaaacgtggccaatatggacaacttcttcgcccccgttttcaccatgggcaaatattatacgcaaggcgacaaggtgctgatgccgctggcgattcaggttcatcatgccgtctgtgatggcttccatgtcggcagaatgcttaatgaattacaacagtactgcgatgagtggcagggcggggcgtaatttttttaaggcagttattggtgcccttaaacgcctggtgctacgcctgaataagtgataataagcggatgaatggcagaaattcgtcgaagcttaacacagaaaaaagcccgcacctgacagtgcgggctttttttttcgaccactgcagtctgttacaggtcactaataccatctaagtagttgattcatagtgactgcatatgttgtgttttacagtattatgtagtctgttttttatgcaaaatctaatttaatatattgatatttatatcattttacgtttctcgttcagcttttttatactaacttgagcgatttacgagacagacactgggagtaaataaagtatg

SEQ ID NO: 40 - DNA, 21 bp, Artificial Sequence
  Primer P21
ccagtaattcagaaatgttgg

SEQ ID NO: 41 - DNA, 21 bp, Artificial Sequence
  Primer P22
ccatattacgaccatgagtgg

SEQ ID NO: 42 - DNA, 1354 bp, Artificial Sequence
  PCR product
ccagtaattcagaaatgttggagaaattatcatgatgcaacatcaggtcaatgtatcggctcgcttcaatccagaaaccttagaacgtgttttacgcgtggtgcgtcatcgtggtttccacgtctgctcaatgaatatggccgccgccagcgatgcacaaaatataaatatcgaattgaccgttgccagcccacggtcggtcgacttactgtttagtcagttaaataaactggtggacgtcgcacacgttgccatctgccagagcacaaccacatcacaacaaatccgcgcctgagcgcaaaaggaatataaaaatgaccacgaagaaagctgattacatttggttcaatggggagatggttcgctgggaagacgcgaaggtgcatgtgatgtcgcacgcgctgcactatggcacttcggtttttgaaggcatccgttgctacgactcgcacaaaggaccggttgtattccgccatcgtgagcatatgcagcgtctgcatgactccgccaaaatctatcgcttcccggtttcgcagagcattgatgagctgatggaagcttgtcgtgacgtgatccgcaaaaacaatctcaccagcgcctatatccgtccgctgatcttcgtcggtgatgttggcatgggagtaaacccgccagcgggatactcaaccgacgtgattatcgctgctttcccgtggggagcgtatctgggcgcagaagcgctggagcaggggatcgatgcgatggtttcctcctggaaccgcgcacgaccaaacaccatcccgacggcggcaaaagccggtggtaactacctctcttccctgctggtgggtagcgaagcgcgccgccacggttatcaggaaggtatcgcgctggatgtgaacggttatatctctgaaggcgcaggcgaaaacctgtttgaagtgaaagatggtgtgctgttcaccccaccgttcacctcctccgcgctgccgggtattacccgtgatgccatcatcaaactggcgaaagagctgggaattgaagtacgtgagcaggtgctgtcgcgcgaatccctgtacctggcggatgaagtgtttatgtccggtacggcggcagaaatcacgccagtgcgcagcgtagacggtattcaggttggcgaaggccgttgtggcccggttaccaaacgcattcagcaagccttcttcggcctcttcactggcgaaaccgaagataaatggggctggttagatcaagttaatcaataaatacaaaaaatgggacggcacgcaccgtcccatttacgagacagacactgggagtaaataaagtatgcctaagtaccgttccgccaccaccactcatggtcgtaatatgg

SEQ ID NO: 43 - DNA, 2015 bp, Artificial Sequence
  PCR product
ccagtaattcagaaatgttggagaaattatcatgatgcaacatcaggtcaatgtatcggctcgcttcaatccagaaaccttagaacgtgttttacgcgtggtgcgtcatcgtggtttccacgtctgctcaatgaatatggccgccgccagcgatgcacaaaatataaatatcgaattgaccgttgccagcccacggtcggtcgacttactgtttagtcagttaaataaactggtggacgtcgcacacgttgccatctgccagagcacaaccacatcacaacaaatccgcgcctgatgaagcctgcttttttatactaagttggcattataaaaaagcattgcttatcaatttgttgcaacgaacaggtcactatcagtcaaaataaaatcattatttgatttcgaattctcatgtttgacagcttatcatcgataagctttaatgcggtagtttatcacagttaaattgctaacgcagtcaggcaccgtgtatgaaatctaacaatgcgctcatcgtcatcctcggcaccgtcaccctggatgctgtaggcataggcttggttatgccggtactgccgggcctcttgcgggatatcgtccattccgacagcatcgccagtcactatggcgtgctgctagcgctatatgcgttgatgcaatttctatgcgcacccgttctcggagcactgtccgaccgctttggccgccgcccagtcctgctcgcttcgctacttggagccactatcgactacgcgatcatggcgaccacacccgtcctgtggatctccggataagtagacagcctgataagtcgcacgaaaaacaggtattgacaacatgaagtaacatgcagtaagatacaaatcgctaggtaacactagcagcgtcaaccgggcgctctagctagagccaagctagcttggccggatccgagattttcaggagctaaggaagctaaaatggagaaaaaaatcactggatataccaccgttgatatatcccaatggcatcgtaaagaacattttgaggcatttcagtcagttgctcaatgtacctataaccagaccgttcagctggatattacggcctttttaaagaccgtaaagaaaaataagcacaagttttatccggcctttattcacattcttgcccgcctgatgaatgctcatccggaattccgtatggcaatgaaagacggtgagctggtgatatgggatagtgttcacccttgttacaccgttttccatgagcaaactgaaacgttttcatcgctctggagtgaataccacgacgatttccggcagtttctacacatatattcgcaagatgtggcgtgttacggtgaaaacctggcctatttccctaaagggtttattgagaatatgtttttcgtctcagccaatccctgggtgagtttcaccagttttgatttaaacgtggccaatatggacaacttcttcgcccccgttttcaccatgggcaaatattatacgcaaggcgacaaggtgctgatgccgctggcgattcaggttcatcatgccgtctgtgatggcttccatgtcggcagaatgcttaatgaattacaacagtactgcgatgagtggcagggcggggcgtaatttttttaaggcagttattggtgcccttaaacgcctggtgctacgcctgaataagtgataataagcggatgaatggcagaaattcgtcgaagcttaacacagaaaaaagcccgcacctgacagtgcgggctttttttttcgaccactgcagtctgttacaggtcactaataccatctaagtagttgattcatagtgactgcatatgttgtgttttacagtattatgtagtctgttttttatgcaaaatctaatttaatatattgatatttatatcattttacgtttctcgttcagcttttttatactaacttgagcgatttacgagacagacactgggagtaaataaagtatgcctaagtaccgttccgccaccaccactcatggtcgtaatatgg

SEQ ID NO: 44 - DNA, 60 bp, Artificial Sequence
  Primer P23
aattttgtttaactttaagaaggagatataatgatcccggacgtatcacaggcgctggcc

SEQ ID NO: 45 - DNA, 55 bp, Artificial Sequence
  Primer P24
atctaagctttctagtcaggcgtgtttttccagccacaccgcaaacggttcggta

SEQ ID NO: 46 - DNA, 100 bp, Artificial Sequence
  Ptac4071f10 fragment
ccctgttgacaattaatcatcggctcgtataatgtgtggaatcgtgagcggataacaatttcacacaaataattttgtttaactttaagaaggagatata

SEQ ID NO: 47 - DNA, 45 bp, Artificial Sequence
  Primer P25
aacttgagcgtctagccctgttgacaattaatcatcggctcgtat

SEQ ID NO: 48 - DNA, 100 bp, Artificial Sequence
  Primer P26
taatgagttatatgcaaattagtaaaattatgttgctatgtcagatagttacgatttagtcatctaactatgaagcctgcttttttatactaagttggca

SEQ ID NO: 49 - DNA, 100 bp, Artificial Sequence
  Primer P27
taataatatccacataaataaaacaacgggcgtgttatacgcccgtttcaatatttaacacatggagagatcaggcgtgtttttccagccacaccgcaaa

SEQ ID NO: 50 - DNA, 35 bp, Artificial Sequence
  Primer P28
gtacccggggatcctttactgctgctgtaaacgtg

SEQ ID NO: 51 - DNA, 35 bp, Artificial Sequence
  Primer P29
gcctgcaggtcgactatgatcaagctcggcatcgt

SEQ ID NO: 52 - DNA, 27 bp, Artificial Sequence
  Primer P30
gacggttttggcggcgcgtcgattttc

SEQ ID NO: 53 - DNA, 27 bp, Artificial Sequence
  Primer P31
gccgccaaaaccgtccagcggcttaag

SEQ ID NO: 54 - DNA, 55 bp, Artificial Sequence
  Primer P32
aattttgtttaactttaagaaggagatataatgatcaagctcggcatcgtgatgg

SEQ ID NO: 55 - DNA, 55 bp, Artificial Sequence
  Primer P33
atctaagctttctagttactgctgctgtaaacgtgcttcgatggcatccattaac

SEQ ID NO: 56 - DNA, 80 bp, Artificial Sequence
  Primer P34
ttaccgcgctacaagtacgatttggcgatttgggctaacggagaagaatatgaagcctgcttttttatactaagttggca

SEQ ID NO: 57 - DNA, 90 bp, Artificial Sequence
  Primer P35
aagggcgctgtcactcagagtctcaacgagatccttctcgctaaggtgggttactgctgctgtaaacgtgcttcgatggcatccattaac

SEQ ID NO: 58 - DNA, 1791 bp, Artificial Sequence
  PCR product
agtttgatcgcgctaaatactgcttcaccacaaggacgctcaagttagtataaaaaagctgaacgagaaacgtaaaatgatataaatatcaatatattaaattagattttgcataaaaaacagactacataatactgtaaaacacaacatatgcagtcactatgaatcaactacttagatggtattagtgacctgtaacagactgcagtggtcgaaaaaaaaagcccgcactgtcaggtgcgggcttttttctgtgttaagcttcgacgaatttctgccattcatccgcttattatcacttattcaggcgtagcaccaggcgtttaagggcaccaataactgccttaaaaaaattacgccccgccctgccactcatcgcagtactgttgtaattcattaagcattctgccgacatggaagccatcacagacggcatgatgaacctgaatcgccagcggcatcagcaccttgtcgccttgcgtataatatttgcccatggtgaaaacgggggcgaagaagttgtccatattggccacgtttaaatcaaaactggtgaaactcacccagggattggctgagacgaaaaacatattctcaataaaccctttagggaaataggccaggttttcaccgtaacacgccacatcttgcgaatatatgtgtagaaactgccggaaatcgtcgtggtattcactccagagcgatgaaaacgtttcagtttgctcatggaaaacggtgtaacaagggtgaacactatcccatatcaccagctcaccgtctttcattgccatacggaattccggatgagcattcatcaggcgggcaagaatgtgaataaaggccggataaaacttgtgcttatttttctttacggtctttaaaaaggccgtaatatccagctgaacggtctggttataggtacattgagcaactgactgaaatgcctcaaaatgttctttacgatgccattgggatatatcaacggtggtatatccagtgatttttttctccattttagcttccttagctcctgaaaatctcggatccgatatctagctagagcgcccggttgacgctgctagtgttacctagcgatttgtatcttactgcatgttacttcatgttgtcaatacctgtttttcgtgcgacttatcaggctgtctacttatccggagatccacaggacgggtgtggtcgccatgatcgcgtagtcgatagtggctccaagtagcgaagcgagcaggactgggcggcggccaaagcggtcggacagtgctccgagaacgggtgcgcatagaaattgcatcaacgcatatagcgctagcagcacgccatagtgactggcgatgctgtcggaatggacgatatcccgcaagaggcccggcagtaccggcataaccaagcctatgcctacagcatccagggtgacggtgccgaggatgacgatgagcgcattgttagatttcatacacggtgcctgactgcgttagcaatttaactgtgataaactaccgcattaaagcttatcgatgataagctgtcaaacatgagaattcgaaatcaaataatgattttattttgactgatagtgacctgttcgttgcaacaaattgataagcaatgcttttttataatgccaacttagtataaaaaagcaggcttcaagatctctcacctaccaaacaatgcccccctgcaaaaaataaattcataaaaaacatacagataaccatctgcggtgataaattatctctggcggtgttgacaattaatcatcggctcgtataatgt

SEQ ID NO: 59 - DNA, 500 bp, Artificial Sequence
  PCR product
tctgctcaatcagcacaacttcatcacgcactgggtcaaagggtagcaagactgcggcgtgaccgcgctcaaaaatttcccgccgcacctcatgactcatttgcccgttgaatagacgatgacgaaatctataaagatctaatgaaaaaaagccgcgataaagtgtttctcgtgcaataatttctacatcgtttttgccaaatgtaacgggcaggttgtctggcttaagcattgttaatgtcctggcactaatagtgaattaaatgtgaatttcagcgacgtttgactgccgtttgagcagtcatgtgttaaattgaggcacattaacgccctatggcacgtaacgccaaccttttgcggtagcggcttctgctagaatccgcaataattttacagtttgatcgcgctaaatactgcttcaccacaaggaatgcaaatgaagaaattgctccccattcttatcggcctgagcctttctgggttcagttcgttgagccagg

SEQ ID NO: 60 - DNA, 2279 bp, Artificial Sequence
  PCR product
tctgctcaatcagcacaacttcatcacgcactgggtcaaagggtagcaagactgcggcgtgaccgcgctcaaaaatttcccgccgcacctcatgactcatttgcccgttgaatagacgatgacgaaatctataaagatctaatgaaaaaaagccgcgataaagtgtttctcgtgcaataatttctacatcgtttttgccaaatgtaacgggcaggttgtctggcttaagcattgttaatgtcctggcactaatagtgaattaaatgtgaatttcagcgacgtttgactgccgtttgagcagtcatgtgttaaattgaggcacattaacgccctatggcacgtaacgccaaccttttgcggtagcggcttctgctagaatccgcaataattttacagtttgatcgcgctaaatactgcttcaccacaaggacgctcaagttagtataaaaaagctgaacgagaaacgtaaaatgatataaatatcaatatattaaattagattttgcataaaaaacagactacataatactgtaaaacacaacatatgcagtcactatgaatcaactacttagatggtattagtgacctgtaacagactgcagtggtcgaaaaaaaaagcccgcactgtcaggtgcgggcttttttctgtgttaagcttcgacgaatttctgccattcatccgcttattatcacttattcaggcgtagcaccaggcgtttaagggcaccaataactgccttaaaaaaattacgccccgccctgccactcatcgcagtactgttgtaattcattaagcattctgccgacatggaagccatcacagacggcatgatgaacctgaatcgccagcggcatcagcaccttgtcgccttgcgtataatatttgcccatggtgaaaacgggggcgaagaagttgtccatattggccacgtttaaatcaaaactggtgaaactcacccagggattggctgagacgaaaaacatattctcaataaaccctttagggaaataggccaggttttcaccgtaacacgccacatcttgcgaatatatgtgtagaaactgccggaaatcgtcgtggtattcactccagagcgatgaaaacgtttcagtttgctcatggaaaacggtgtaacaagggtgaacactatcccatatcaccagctcaccgtctttcattgccatacggaattccggatgagcattcatcaggcgggcaagaatgtgaataaaggccggataaaacttgtgcttatttttctttacggtctttaaaaaggccgtaatatccagctgaacggtctggttataggtacattgagcaactgactgaaatgcctcaaaatgttctttacgatgccattgggatatatcaacggtggtatatccagtgatttttttctccattttagcttccttagctcctgaaaatctcggatccgatatctagctagagcgcccggttgacgctgctagtgttacctagcgatttgtatcttactgcatgttacttcatgttgtcaatacctgtttttcgtgcgacttatcaggctgtctacttatccggagatccacaggacgggtgtggtcgccatgatcgcgtagtcgatagtggctccaagtagcgaagcgagcaggactgggcggcggccaaagcggtcggacagtgctccgagaacgggtgcgcatagaaattgcatcaacgcatatagcgctagcagcacgccatagtgactggcgatgctgtcggaatggacgatatcccgcaagaggcccggcagtaccggcataaccaagcctatgcctacagcatccagggtgacggtgccgaggatgacgatgagcgcattgttagatttcatacacggtgcctgactgcgttagcaatttaactgtgataaactaccgcattaaagcttatcgatgataagctgtcaaacatgagaattcgaaatcaaataatgattttattttgactgatagtgacctgttcgttgcaacaaattgataagcaatgcttttttataatgccaacttagtataaaaaagcaggcttcaagatctctcacctaccaaacaatgcccccctgcaaaaaataaattcataaaaaacatacagataaccatctgcggtgataaattatctctggcggtgttgacaattaatcatcggctcgtataatgtgtggaattgtgataaggaggtgatatgcaaatgaagaaattgctccccattcttatcggcctgagcctttctgggttcagttcgttgagccagg

SEQ ID NO: 61 - DNA, 60 bp, Artificial Sequence
  Primer P36
agtttgatcgcgctaaatactgcttcaccacaaggacgctcaagttagtataaaaaagct

SEQ ID NO: 62 - DNA, 70 bp, Artificial Sequence
  Primer P37
gccgataagaatggggagcaatttcttcatttgcatatcacctccttatcacaattccacacattatacg

SEQ ID NO: 63 - DNA, 20 bp, Artificial Sequence
  Primer P38
tctgctcaatcagcacaact

SEQ ID NO: 64 - DNA, 19 bp, Artificial Sequence
  Primer P39
cctggctcaacgaactgaa